European Patent Specification EP 3 452 513 B1, published April 17, 2024. Title: Humanized anti-IL-1R3 antibodies. Applicant: MAB Discovery GmbH. The sequence listing filed with the application follows.

SEQUENCE LISTING (175 sequences)

SEQ ID NO: 1 - protein, 118 aa, Artificial Sequence
  humanized antibody
EVQLEESGGGLVQPGGSLRLSCAASGFSFSSSYWICWVRQAPGKGLEWVSCIYTGSGGTYYASWEKGRFTISRDNSKNTLYLQMNSLRAEDTAVYFCARDPGYSSWLWGQGTLVTVSS

SEQ ID NO: 2 - protein, 122 aa, Artificial Sequence
  humanized antibody
EVQLEESGGDLVQPGGSLRLSCAASGFSFSSSHYMCWVRQAPGKGLEWVSCIYAGSSGNTYYANWAKGRFTISRDNSKNTLYLQMNSLRAEDTAVYFCARVDASSSGSWDLWGQGTLVTVSS

SEQ ID NO: 3 - protein, 123 aa, Artificial Sequence
  humanized antibody
EVQLEESGGRLVQPGGSLRLSCAVSGIDLSSYAMGWVRQAPGKGLEYVSVITSSATTYYASWAKGRFTISRDNSKNTLYLQMNSLRAEDTAVYFCARGGPGYSTNTHYAFDPWGQGTLVTVSS

SEQ ID NO: 4 - protein, 119 aa, Artificial Sequence
  humanized antibody
EVQLEESGGRVVQPGRSLRLSCAVSGIDLDNYAMGWVRQAPGKGLEYVAVISSDGFFYDASWAKGRFTISRDNSKNTLYLQMNSLRAEDTAVYFCARDRGTSTGSLDLWGQGTLVTVSS

SEQ ID NO: 5 - protein, 125 aa, Artificial Sequence
  humanized antibody
EVQLEESGGRLVQPGGSLRLSCAASGFSLSSYYMSWVRQAPGKGLEWVSIISGSASTYYATWAKGRFTISRDNSKNTLYLQMNSLRAEDTAVYFCARTHYAAVAGYGYASRLDLWGQGTLVTVSS

SEQ ID NO: 6 - protein, 120 aa, Artificial Sequence
  humanized antibody
EVQLEESGGDLVQPGGSLRLSCAASGFSFSSNYWICWVRQAPGKGLELVSCIYTSTGNTWYASWAKGRFTISRDNSKNTLYLQMNSLRAEDTAVYFCARDLLVVTSFNLWGQGTLVTVSS

SEQ ID NO: 7 - protein, 120 aa, Artificial Sequence
  humanized antibody
EVQLEESGGDLVQPGGSLRLSCAASGFSFSSSYYMCWVRQAPGKGLEWVSCIYAGSSGVTYYASWAKGRFTISRDNSKNTLYLQMNSLRAEDTAVYFCASETDGNYFNLWGQGTLVTVSS

SEQ ID NO: 8 - protein, 120 aa, Artificial Sequence
  humanized antibody
EVQLEQSGGGLVQPGGSLRLSCAASGFSLSTSYWRCWVRQAPGKGLEWVSCIYAGSGDVTYYANWVNGRFTISRDNSKNTLYLQMNSLRAEDTAVYYCASGVGFGYFNLWGQGTLVTVSS

SEQ ID NO: 9 - protein, 122 aa, Artificial Sequence
  humanized antibody
EVQLEESGGGLVQPGGSLRLSCAASGIDFSSYYYMCWVRQAPGKGLEWVSCIFIGYGDVTWYASWAKGRFTISRDNSKNTLYLQMNSLRAEDTAVYFCARALGSSGYRVNLWGQGTLVTVSS

SEQ ID NO: 10 - protein, 115 aa, Artificial Sequence
  humanized antibody
EVQLEESGGRLVQPGGSLRLSCAASGFSLSSYWMSWVRQAPGKGLEWVSMIYGSGYTYYASWAKGRFTISRDNSKNTLYLQMNSLRAEDTAVYFCARDPQYFILWGQGTLVTVSS

SEQ ID NO: 11 - protein, 120 aa, Artificial Sequence
  humanized antibody
EVQLEESGGRLVQPGGSLRLSCAVSGFSLSSYDMSWVRQAPGKGLEWVSTIYIGGTTAYASWPKGRFTISRDNSKNTLYLQMNSLRAEDTAVYFCARLQGANYYNSLALWGQGTLVTVSS

SEQ ID NO: 12 - protein, 120 aa, Artificial Sequence
  humanized antibody
EVQLVESGGGLVQPGGSLRLSCAASGFDFSSNYYMCWVRQAPGKGLELVSCIYTNSGNTWSASWAKGRFTISRDNSKNTLYLQMNSLRAEDTAVYFCARDLNYPDTSNLWGQGTLVTVSS

SEQ ID NO: 13 - protein, 119 aa, Artificial Sequence
  humanized antibody
EVQLEESGGDLVQPGGSLRLSCAASGFSFSFGYYMCWVRQAPGKGLEWVSCIYGDSSDTLYANWAKGRFTISRDNSKNTLYLQMNSLRAEDTAVYFCARYPGGSYYNLWGQGTLVTVSS

SEQ ID NO: 14 - protein, 122 aa, Artificial Sequence
  humanized antibody
EVQLEESGGDLVQPGGSLRLSCAASGFSFSSTYYMCWVRQAPGKGLEWVSCIYAGSSGSTYYASWAKGRFTISRDNSKNTLYLQMNSLRAEDTAVYFCARVDGSSSGSWDLWGQGTLVTVSS

SEQ ID NO: 15 - protein, 122 aa, Artificial Sequence
  humanized antibody
EVQLEESGGDLVQPGGSLRLSCAASGISFSSSDFMCWVRQAPGKGLEWVSCIYAGSSVSIYYATWAKGRFTISRDNSKNTLYLQMNSLRAEDTAVYFCARSTGSVGRGFNLWGQGTLVTVSS

SEQ ID NO: 16 - protein, 121 aa, Artificial Sequence
  humanized antibody
EVQLVESGGGLVQPGGSLRLSCAASGFSFSSIYYMCWVRQAPGKGLEWVSCIYTGNSDFTYYANWAKGRFTISRDNSKNTLYLQMNSLRAEDTAVYFCARFRDDYASLKLWGQGTLVTVSS

SEQ ID NO: 17 - protein, 120 aa, Artificial Sequence
  humanized antibody
EVQLEESGGGLVQPGGSLRLSCAASGFSFSSGYDMCWVRQAPGKGLEWVSCIYTGSGSTYYANWAKGRFTISRDNSKNTLYLQMNSLRAEDTAVYFCARNSNDWMYFNLWGQGTLVTVSS

SEQ ID NO: 18 - protein, 117 aa, Artificial Sequence
  humanized antibody
EVQLEQSGGGLVQPGGSLRLSCAASGFSFSSSYWICWVRQAPGKGLEWVACIYTGSGGTYYASWEKGRFTISKTSSTTLYLQMNSLRAEDTAVYFCARDPGYSSWLWGQGTLVTVSS

SEQ ID NO: 19 - protein, 122 aa, Artificial Sequence
  humanized antibody
EVQLEESGGDLVQPGASLRLSCAASGFSFSSSHYMCWVRQAPGKGLEWVACIYAGSSGNTYYANWAKGRFTISKTNSKNTLYLQMNSLRAEDTAVYFCARVDASSSGSWDLWGQGTLVTVSS

SEQ ID NO: 20 - protein, 122 aa, Artificial Sequence
  humanized antibody
EVQLLESGGRLVQPGTSLRLSCAVSGIDLSSYAMGWVRQAPGKGLEYVGVITSSATTYYASWAKGRFTISKTSSTTLYLQMNSLRAEDTAVYFCARGGPGYSTNTHYAFDPWGQGTLVTVSS

SEQ ID NO: 21 - protein, 119 aa, Artificial Sequence
  humanized antibody
EVQLEESGGRVVQPGTSLRLSCAVSGIDLDNYAMGWVRQAPGKGLEYVAVISSDGFFYDASWAKGRFTISKANSKNTLYLQMNSLRAEDTAVYFCARDRGTSTGSLDLWGQGTLVTVSS

SEQ ID NO: 22 - protein, 123 aa, Artificial Sequence
  humanized antibody
QVQLEESGGRLVQPGTSLRLSCAASGFSLSSYYMSWVRQAPGKGLEWVAIISGSASTYYATWAKGRFTISKTSTTLYLQMNSLRAEDTAVYFCARTHYAAVAGYGYASRLDLWGQGTLVTVSS

SEQ ID NO: 23 - protein, 120 aa, Artificial Sequence
  humanized antibody
QVQLQESGGDLVQPGGSLRLSCAASGFSFSSNYWICWVRQAPGKGLELVACIYTSTGNTWYASWAKGRFTISRDNSKNTLYLQMNSLRAEDTAVYFCARDLLVVTSFNLWGQGTLVTVSS

SEQ ID NO: 24 - protein, 119 aa, Artificial Sequence
  humanized antibody
EVQLVESGGDLVQPGASLRLSCAASGFSFSSSYYMCWVRQAPGKGLEWVACIYAGSSGVTYYASWAKGRFTISDTSSTTLYLQMNSLRAEDTAVYFCASETDGNYFNLWGQGTLVTVSS

SEQ ID NO: 25 - protein, 120 aa, Artificial Sequence
  humanized antibody
EVQLEQSGGGLVQPGGSLRLSCAASGFSLSTSYWRCWVRQAPGKGLEWVACIYAGSGDVTYYANWVNGRFTISRDNSKSTLYLQMNSLRAEDTAVYYCASGVGFGYFNLWGQGTLVTVSS

SEQ ID NO: 26 - protein, 122 aa, Artificial Sequence
  humanized antibody
EVQLEESGGGLVQPGGSLRLSCAASGIDFSSYYYMCWVRQAPGKGLEWVACIFIGYGDVTWYASWAKGRFTISKANSKNTLYLQMNSLRAEDTAVYFCARALGSSGYRVNLWGQGTLVTVSS

SEQ ID NO: 27 - protein, 113 aa, Artificial Sequence
  humanized antibody
QVQLEESGGRLVQPGASLRLSCAASGFSLSSYWMSWVRQAPGKGLEWVAMIYGSGYTYYASWAKGRFTISTTSTTLYLQMNSLRAEDTAVYFCARDPQYFILWGQGTLVTVSS

SEQ ID NO: 28 - protein, 120 aa, Artificial Sequence
  humanized antibody
EVQLEESGGRLVQPGTSLRLSCAVSGFSLSSYDMSWVRQAPGKGLEWVSTIYIGGTTAYASWPKGRFTISKTNSKNTLYLQMNSLRAEDTAVYFCARLQGANYYNSLALWGQGTLVTVSS

SEQ ID NO: 29 - protein, 119 aa, Artificial Sequence
  humanized antibody
QVQLVESGGGLVQPGGSLRLSCAASGFDFSSNYYMCWVRQAPGKGLELVACIYTNSGNTWSASWAKGRFTISKTNSTTLYLQMNSLRAEDTAVYFCARDLNYPDTSNLWGQGTLVTVSS

SEQ ID NO: 30 - protein, 119 aa, Artificial Sequence
  humanized antibody
EVQLEESGGDLVQPGGSLRLSCAASGFSFSFGYYMCWVRQAPGKGLEWVACIYGDSSDTLYANWAKGRFTISKTNSKNTLYLQMNSLRAEDTAVYFCARYPGGSYYNLWGQGTLVTVSS

SEQ ID NO: 31 - protein, 120 aa, Artificial Sequence
  humanized antibody
QVQLQESGGDLVQPGASLRLSCAASGFSFSSTYYMCWVRQAPGKGLEWVACIYAGSSGSTYYASWAKGRFTISKNSSTLYLQMNSLRAEDTAVYFCARVDGSSSGSWDLWGQGTLVTVSS

SEQ ID NO: 32 - protein, 121 aa, Artificial Sequence
  humanized antibody
EVQLEESGGDLVQPGASLRLSCAASGISFSSSDFMCWVRQAPGKGLEWVACIYAGSSVSIYYATWAKGRFTISKASSTTLYLQMNSLRAEDTAVYFCARSTGSVGRGFNLWGQGTLVTVSS

SEQ ID NO: 33 - protein, 121 aa, Artificial Sequence
  humanized antibody
EVQLVESGGGLVQPGGSLRLSCAASGFSFSSIYYMCWVRQAPGKGLEWVGCIYTGNSDFTYYANWAKGRFTISRDNSKSTLYLQMNSLRAEDTAVYFCARFRDDYASLKLWGQGTLVTVSS

SEQ ID NO: 34 - protein, 120 aa, Artificial Sequence
  humanized antibody
QVQLQESGGGLVQPGGSLRLSCTASGFSFSSGYDMCWVRQAPGKGLEWVGCIYTGSGSTYYANWAKGRFTISKDNSKTTLYLQMNSLRAEDTAVYFCARNSNDWMYFNLWGQGTLVTVSS

SEQ ID NO: 35 - protein, 110 aa, Artificial Sequence
  humanized antibody
DIVMTQSPSSLSASVGDRVTITCQASESISNYLSWYQQKPGQAPKLLIYLASTLASGVPSRFSGSGSGTDFTLTISSLQPEDFATYYCQNWWVIEHNGAAFGGGTKVVIK

SEQ ID NO: 36 - protein, 110 aa, Artificial Sequence
  humanized antibody
DIQMTQSPSSLSASVGDRVTITCQASESIYSNLAWYQQKPGQAPKLLIYAASLLASGVPSRFSGSGSGTDFTLTISSLQPEDFATYYCQSASYSTGPDWTFGQGTKVVIK

SEQ ID NO: 37 - protein, 110 aa, Artificial Sequence
  humanized antibody
DIQMTQSPSSLSASVGDRVTITCQASQSIYIYLSWYQQKPGQAPKLLIYDASKLASGVPSRFSGSGSGTDFTLTISSLQPEDFATYYCQQGATTYNVDNVFGQGTKVVIK

SEQ ID NO: 38 - protein, 111 aa, Artificial Sequence
  humanized antibody
DIVMTQSPSSLSASVGDRVTITCQASENIGNGLAWYQQKPGQAPKLLIYGASTLASGVPSRFSGSGSGTDFTLTISSLQPEDFATYYCQCTYWNPDYIGGAFGGGTKVVIK

SEQ ID NO: 39 - protein, 110 aa, Artificial Sequence
  humanized antibody
DIQMTQSPSSLSASVGDRVTITCLASEDIYSGISWYQQKPGKAPKLLIYAASNLESGVPSRFSGSGSGTDFTLTISSLQPEDFATYYCLGGYSYSNTGPTFGQGTKVEIK

SEQ ID NO: 40 - protein, 113 aa, Artificial Sequence
  humanized antibody
DIVMTQSPSSLSASVGDRVTITCQASEDIYSNLAWFQQKPGQAPKLLIYGASTLASGVPSRFSGSGSGTEFTLTISSLQPEDFATYYCLGVCTDISTDDLYNAFGQGTKVVIK

SEQ ID NO: 41 - protein, 110 aa, Artificial Sequence
  humanized antibody
DIVMTQSPSSLSASVGDRVTITCQASEDIYSNLAWFQQKPGQAPKLLIYRASTLASGVPSRFSGSGSGTEFTLTISSLQPEDFATYYCLGVYTYSTDIHAFGGGTKVVIK

SEQ ID NO: 42 - protein, 110 aa, Artificial Sequence
  humanized antibody
DIVMTQSPSSLSASVGDRVTITCQASEDIYSNLAWFQQKPGQAPKLLIYDASTLASGVPSRFSGSGSGTEFTLTISSLQPEDFATYYCLGVYTHISADNAFGGGTKVVIK

SEQ ID NO: 43 - protein, 111 aa, Artificial Sequence
  humanized antibody
DIQMTQSPSSLSASVGDRVTITCQASENIYSSLAWYQQKPGQAPKLLIYDASDLASGVPSRFSGSGSGTDFTLTISSLQPEDFATYYCQQGYYSGGTDNDVFGGGTKVVIK

SEQ ID NO: 44 - protein, 112 aa, Artificial Sequence
  humanized antibody
DIVMTQSPSSLSASVGDRVTITCQSSQSVDGNNLLSWYQQKPGQAPKLLIYDASNLASGVPSRFSGSGSGTDFTLTISSLQPEDFATYYCQGSYYSSSWYNVFGQGTKVVIK

SEQ ID NO: 45 - protein, 108 aa, Artificial Sequence
  humanized antibody
DIQMTQSPSSLSASVGDRVTITCQASQSIYSFLSWYQQKPGQAPKLLIYAASDLESGVPSRFSGSGSGTDFTLTISSLQPEDFATYYCQCNYIIDYGAFGQGTKVVIK

SEQ ID NO: 46 - protein, 108 aa, Artificial Sequence
  humanized antibody
DIQMTQSPSSLSASVGDRVTITCQASQSIGYYLAWYQQKPGQAPKLLIYRASTLASGVPSRFSGSGSGTDFTLTISSLQPEDFATYYCQSYYNSDSDAFGQGTKVVIK

SEQ ID NO: 47 - protein, 110 aa, Artificial Sequence
  humanized antibody
DIVMTQSPSSLSASVGDRVTITCQASQTISINLAWYQQKPGQAPKLLIYYASTLASGVPSRFSGSGSGTDFTLTISSLQPEDFATYYCQQGYTEDNIDNTFGQGTKVVIK

SEQ ID NO: 48 - protein, 110 aa, Artificial Sequence
  humanized antibody
DIQMTQSPSSLSASVGDRVTITCQASQNIYSNLAWYQQKPGQAPKLLIYAASLLASGVPSRFSGSGSGTDFTLTISSLQPEDFATYYCQGAVYSGNTEWAFGQGTKVVIK

SEQ ID NO: 49 - protein, 113 aa, Artificial Sequence
  humanized antibody
DIVMTQSPSSLSASVGDRVTITCQASQSVYNSNHLSWYQQKPGQAPKLLIYSASTLASGVPSRFSGSGSGTDFTLTISSLQPEDFATYYCQGEFSCVSADCIAFGGGTKVVIK

SEQ ID NO: 50 - protein, 110 aa, Artificial Sequence
  humanized antibody
DIQMTQSPSSLSASVGDRVTITCQASQSISSYLSWYQQKPGQAPKLLIYGASNLASGVPSRFSGSGSGTDFTLTISSLQPEDFATYYCQCTYYDNNYGGAFGGGTKVVIK

SEQ ID NO: 51 - protein, 114 aa, Artificial Sequence
  humanized antibody
DIVMTQSPSSLSASVGDRVTITCQASESISANYWSWYQQKPGQAPKLLIYGASTLASGVPSRFSGSGSGTDFTLTISSLQPEDFATYFCQSWYYSGSGSYHSWAFGQGTKVVIK

SEQ ID NO: 52 - protein, 110 aa, Artificial Sequence; identical to SEQ ID NO: 35
  humanized antibody

SEQ ID NO: 53 - protein, 110 aa, Artificial Sequence
  humanized antibody
AIQMTQSPSSLSASVGDRVTITCQASESIYSNLAWYQQKPGQAPKLLIYAASLLASGVPSRFSGSGSGTDYTLTISSLQPEDFATYYCQSASYSTGPDWTFGQGTKVVIK

SEQ ID NO: 54 - protein, 110 aa, Artificial Sequence
  humanized antibody
AIRMTQSPSSLSASVGDRVTITCQASQSIYIYLSWYQQKPGQAPKLLIYDASKLASGVPSRFSGSGSGTDFTLTISSLQPEDFATYYCQQGATTYNVDNVFGQGTKVVIK

SEQ ID NO: 55 - protein, 111 aa, Artificial Sequence
  humanized antibody
ELVMTQSPSSLSASVGDRVTITCQASENIGNGLAWYQQKPGQAPKLLIYGASTLASGVPSRFSGSGSGTDFTLTISSLQPEDFATYYCQCTYWNPDYIGGAFGGGTKVVIK

SEQ ID NO: 56 - protein, 110 aa, Artificial Sequence
  humanized antibody
AIQMTQSPSSLSASVGDRVTITCLASEDIYSGISWYQQKPGKAPKLLIYAASNLESGVPSRFSGSGSGTDYTLTISSLQPEDFATYYCLGGYSYSNTGPTFGQGTKVEIK

SEQ ID NO: 57 - protein, 113 aa, Artificial Sequence; identical to SEQ ID NO: 40
  humanized antibody

SEQ ID NO: 58 - protein, 110 aa, Artificial Sequence; identical to SEQ ID NO: 41
  humanized antibody

SEQ ID NO: 59 - protein, 110 aa, Artificial Sequence
  humanized antibody
ELVMTQSPSSLSASVGDRVTITCQASEDIYSNLAWFQQKPGQAPKLLIYDASTLASGVPSRFSGSGSGTEFTLTISSLQPEDFATYYCLGVYTHISADNAFGGGTKVEIK

SEQ ID NO: 60 - protein, 111 aa, Artificial Sequence
  humanized antibody
ALQMTQSPSSLSASVGDRVTITCQASENIYSSLAWYQQKPGQAPKLLIYDASDLASGVPSRFSGSGSGTDFTLTISSLQPEDFATYYCQQGYYSGGTDNDVFGGGTKVVIK

SEQ ID NO: 61 - protein, 112 aa, Artificial Sequence
  humanized antibody
NIVMTQSPSSLSASVGDRVTITCQSSQSVDGNNLLSWYQQKPGQAPKLLIYDASNLASGVPSRFSGSGSGTDFTLTISSLQPEDFATYYCQGSYYSSSWYNVFGQGTKVVIK

SEQ ID NO: 62 - protein, 108 aa, Artificial Sequence
  humanized antibody
DVQMTQSPSSLSASVGDRVTITCQASQSIYSFLSWYQQKPGQAPKLLIYAASDLESGVPSRFSGSGSGTDFTLTISSLQPEDFATYYCQCNYIIDYGAFGQGTKVVIK

SEQ ID NO: 63 - protein, 108 aa, Artificial Sequence; identical to SEQ ID NO: 46
  humanized antibody

SEQ ID NO: 64 - protein, 110 aa, Artificial Sequence
  humanized antibody
AIVMTQSPSSLSASVGDRVTITCQASQTISINLAWYQQKPGQAPKLLIYYASTLASGVPSRFSGSGSGTDFTLTISSLQPEDFATYYCQQGYTEDNIDNTFGQGTKVVIK

SEQ ID NO: 65 - protein, 110 aa, Artificial Sequence
  humanized antibody
AIQMTQSPSSLSASVGDRVTITCQASQNIYSNLAWYQQKPGQAPKLLIYAASLLASGVPSRFSGSGSGTDYTLTISSLQPEDFATYYCQGAVYSGNTEWAFGQGTKVVIK

SEQ ID NO: 66 - protein, 113 aa, Artificial Sequence; identical to SEQ ID NO: 49
  humanized antibody

SEQ ID NO: 67 - protein, 110 aa, Artificial Sequence
  humanized antibody
DVVMTQSPSSLSASVGDRVTITCQASQSISSYLSWYQQKPGQAPKLLIYGASNLASGVPSRFSGSGSGTDFTLTISSLQPEDFATYYCQCTYYDNNYGGAFGGGTKVEIK

SEQ ID NO: 68 - protein, 114 aa, Artificial Sequence; identical to SEQ ID NO: 51
  humanized antibody

SEQ ID NO: 69 - protein, 6 aa, Artificial Sequence
  humanized antibody
SSYWIC

SEQ ID NO: 70 - protein, 6 aa, Artificial Sequence
  humanized antibody
SSHYMC

SEQ ID NO: 71 - protein, 5 aa, Artificial Sequence
  humanized antibody
SYAMG

SEQ ID NO: 72 - protein, 5 aa, Artificial Sequence
  humanized antibody
NYAMG

SEQ ID NO: 73 - protein, 5 aa, Artificial Sequence
  humanized antibody
SYYMS

SEQ ID NO: 74 - protein, 6 aa, Artificial Sequence
  humanized antibody
SNYWIC

SEQ ID NO: 75 - protein, 6 aa, Artificial Sequence
  humanized antibody
SSYYMC

SEQ ID NO: 76 - protein, 6 aa, Artificial Sequence
  humanized antibody
TSYWRC

SEQ ID NO: 77 - protein, 6 aa, Artificial Sequence
  humanized antibody
SYYYMC

SEQ ID NO: 78 - protein, 5 aa, Artificial Sequence
  humanized antibody
SYWMS

SEQ ID NO: 79 - protein, 5 aa, Artificial Sequence
  humanized antibody
SYDMS

SEQ ID NO: 80 - protein, 6 aa, Artificial Sequence
  humanized antibody
SNYYMC

SEQ ID NO: 81 - protein, 6 aa, Artificial Sequence
  humanized antibody
FGYYMC

SEQ ID NO: 82 - protein, 6 aa, Artificial Sequence
  humanized antibody
STYYMC

SEQ ID NO: 83 - protein, 6 aa, Artificial Sequence
  humanized antibody
SSDFMC

SEQ ID NO: 84 - protein, 6 aa, Artificial Sequence
  humanized antibody
SIYYMC

SEQ ID NO: 85 - protein, 6 aa, Artificial Sequence
  humanized antibody
SGYDMC

SEQ ID NO: 86 - protein, 17 aa, Artificial Sequence
  humanized antibody
CIYTGSGGTYYASWEKG

SEQ ID NO: 87 - protein, 18 aa, Artificial Sequence
  humanized antibody
CIYAGSSGNTYYANWAKG

SEQ ID NO: 88 - protein, 16 aa, Artificial Sequence
  humanized antibody
VITSSATTYYASWAKG

SEQ ID NO: 89 - protein, 16 aa, Artificial Sequence
  humanized antibody
VISSDGFFYDASWAKG

SEQ ID NO: 90 - protein, 16 aa, Artificial Sequence
  humanized antibody
IISGSASTYYATWAKG

SEQ ID NO: 91 - protein, 17 aa, Artificial Sequence
  humanized antibody
CIYTSTGNTWYASWAKG

SEQ ID NO: 92 - protein, 18 aa, Artificial Sequence
  humanized antibody
CIYAGSSGVTYYASWAKG

SEQ ID NO: 93 - protein, 18 aa, Artificial Sequence
  humanized antibody
CIYAGSGDVTYYANWVNG

SEQ ID NO: 94 - protein, 18 aa, Artificial Sequence
  humanized antibody
CIFIGYGDVTWYASWAKG

SEQ ID NO: 95 - protein, 16 aa, Artificial Sequence
  humanized antibody
MIYGSGYTYYASWAKG

SEQ ID NO: 96 - protein, 16 aa, Artificial Sequence
  humanized antibody
TIYIGGTTAYASWPKG

SEQ ID NO: 97 - protein, 17 aa, Artificial Sequence
  humanized antibody
CIYTNSGNTWSASWAKG

SEQ ID NO: 98 - protein, 17 aa, Artificial Sequence
  humanized antibody
CIYGDSSDTLYANWAKG

SEQ ID NO: 99 - protein, 18 aa, Artificial Sequence
  humanized antibody
CIYAGSSGSTYYASWAKG

SEQ ID NO: 100 - protein, 18 aa, Artificial Sequence
  humanized antibody
CIYAGSSVSIYYATWAKG

SEQ ID NO: 101 - protein, 18 aa, Artificial Sequence
  humanized antibody
CIYTGNSDFTYYANWAKG

SEQ ID NO: 102 - protein, 17 aa, Artificial Sequence
  humanized antibody
CIYTGSGSTYYANWAKG

SEQ ID NO: 103 - protein, 8 aa, Artificial Sequence
  humanized antibody
DPGYSSWL

SEQ ID NO: 104 - protein, 11 aa, Artificial Sequence
  humanized antibody
VDASSSGSWDL

SEQ ID NO: 105 - protein, 15 aa, Artificial Sequence
  humanized antibody
GGPGYSTNTHYAFDP

SEQ ID NO: 106 - protein, 11 aa, Artificial Sequence
  humanized antibody
DRGTSTGSLDL

SEQ ID NO: 107 - protein, 17 aa, Artificial Sequence
  humanized antibody
THYAAVAGYGYASRLDL

SEQ ID NO: 108 - protein, 10 aa, Artificial Sequence
  humanized antibody
DLLVVTSFNL

SEQ ID NO: 109 - protein, 9 aa, Artificial Sequence
  humanized antibody
ETDGNYFNL

SEQ ID NO: 110 - protein, 9 aa, Artificial Sequence
  humanized antibody
GVGFGYFNL

SEQ ID NO: 111 - protein, 11 aa, Artificial Sequence
  humanized antibody
ALGSSGYRVNL

SEQ ID NO: 112 - protein, 7 aa, Artificial Sequence
  humanized antibody
DPQYFIL

SEQ ID NO: 113 - protein, 12 aa, Artificial Sequence
  humanized antibody
LQGANYYNSLAL

SEQ ID NO: 114 - protein, 10 aa, Artificial Sequence
  humanized antibody
DLNYPDTSNL

SEQ ID NO: 115 - protein, 9 aa, Artificial Sequence
  humanized antibody
YPGGSYYNL

SEQ ID NO: 116 - protein, 11 aa, Artificial Sequence
  humanized antibody
VDGSSSGSWDL

SEQ ID NO: 117 - protein, 11 aa, Artificial Sequence
  humanized antibody
STGSVGRGFNL

SEQ ID NO: 118 - protein, 10 aa, Artificial Sequence
  humanized antibody
FRDDYASLKL

SEQ ID NO: 119 - protein, 10 aa, Artificial Sequence
  humanized antibody
NSNDWMYFNL

SEQ ID NO: 120 - protein, 11 aa, Artificial Sequence
  humanized antibody
QASESISNYLS

SEQ ID NO: 121 - protein, 11 aa, Artificial Sequence
  humanized antibody
QASESIYSNLA

SEQ ID NO: 122 - protein, 11 aa, Artificial Sequence
  humanized antibody
QASQSIYIYLS

SEQ ID NO: 123 - protein, 11 aa, Artificial Sequence
  humanized antibody
QASENIGNGLA

SEQ ID NO: 124 - protein, 11 aa, Artificial Sequence
  humanized antibody
LASEDIYSGIS

SEQ ID NO: 125 - protein, 11 aa, Artificial Sequence
  humanized antibody
QASEDIYSNLA

SEQ ID NO: 126 - protein, 11 aa, Artificial Sequence
  humanized antibody
QASEDIYSNLA

SEQ ID NO: 127 - protein, 11 aa, Artificial Sequence
  humanized antibody
QASEDIYSNLA

SEQ ID NO: 128 - protein, 11 aa, Artificial Sequence
  humanized antibody
QASENIYSSLA

SEQ ID NO: 129 - protein, 13 aa, Artificial Sequence
  humanized antibody
QSSQSVDGNNLLS

SEQ ID NO: 130 - protein, 11 aa, Artificial Sequence
  humanized antibody
QASQSIYSFLS

SEQ ID NO: 131 - protein, 11 aa, Artificial Sequence
  humanized antibody
QASQSIGYYLA

SEQ ID NO: 132 - protein, 11 aa, Artificial Sequence
  humanized antibody
QASQTISINLA

SEQ ID NO: 133 - protein, 11 aa, Artificial Sequence
  humanized antibody
QASQNIYSNLA

SEQ ID NO: 134 - protein, 13 aa, Artificial Sequence
  humanized antibody
QASQSVYNSNHLS

SEQ ID NO: 135 - protein, 11 aa, Artificial Sequence
  humanized antibody
QASQSISSYLS

SEQ ID NO: 136 - protein, 12 aa, Artificial Sequence
  humanized antibody
QASESISANYWS

SEQ ID NO: 137 - protein, 7 aa, Artificial Sequence
  humanized antibody
LASTLAS

SEQ ID NO: 138 - protein, 7 aa, Artificial Sequence
  humanized antibody
AASLLAS

SEQ ID NO: 139 - protein, 7 aa, Artificial Sequence
  humanized antibody
DASKLAS

SEQ ID NO: 140 - protein, 7 aa, Artificial Sequence
  humanized antibody
GASTLAS

SEQ ID NO: 141 - protein, 7 aa, Artificial Sequence
  humanized antibody
AASNLES

SEQ ID NO: 142 - protein, 7 aa, Artificial Sequence
  humanized antibody
GASTLAS

SEQ ID NO: 143 - protein, 7 aa, Artificial Sequence
  humanized antibody
RASTLAS

SEQ ID NO: 144 - protein, 7 aa, Artificial Sequence
  humanized antibody
DASTLAS

SEQ ID NO: 145 - protein, 7 aa, Artificial Sequence
  humanized antibody
DASDLAS

SEQ ID NO: 146 - protein, 7 aa, Artificial Sequence
  humanized antibody
DASNLAS

SEQ ID NO: 147 - protein, 7 aa, Artificial Sequence
  humanized antibody
AASDLES

SEQ ID NO: 148 - protein, 7 aa, Artificial Sequence
  humanized antibody
RASTLAS

SEQ ID NO: 149 - protein, 7 aa, Artificial Sequence
  humanized antibody
YASTLAS

SEQ ID NO: 150 - protein, 7 aa, Artificial Sequence
  humanized antibody
AASLLAS

SEQ ID NO: 151 - protein, 7 aa, Artificial Sequence
  humanized antibody
SASTLAS

SEQ ID NO: 152 - protein, 7 aa, Artificial Sequence
  humanized antibody
GASNLAS

SEQ ID NO: 153 - protein, 7 aa, Artificial Sequence
  humanized antibody
GASTLAS

SEQ ID NO: 154 - protein, 12 aa, Artificial Sequence
  humanized antibody
QNWWVIEHNGAA

SEQ ID NO: 155 - protein, 12 aa, Artificial Sequence
  humanized antibody
QSASYSTGPDWT

SEQ ID NO: 156 - protein, 12 aa, Artificial Sequence
  humanized antibody
QQGATTYNVDNV

SEQ ID NO: 157 - protein, 13 aa, Artificial Sequence
  humanized antibody
QCTYWNPDYIGGA

SEQ ID NO: 158 - protein, 12 aa, Artificial Sequence
  humanized antibody
LGGYSYSNTGPT

SEQ ID NO: 159 - protein, 15 aa, Artificial Sequence
  humanized antibody
LGVCTDISTDDLYNA

SEQ ID NO: 160 - protein, 12 aa, Artificial Sequence
  humanized antibody
LGVYTYSTDIHA

SEQ ID NO: 161 - protein, 12 aa, Artificial Sequence
  humanized antibody
LGVYTHISADNA

SEQ ID NO: 162 - protein, 13 aa, Artificial Sequence
  humanized antibody
QQGYYSGGTDNDV

SEQ ID NO: 163 - protein, 12 aa, Artificial Sequence
  humanized antibody
QGSYYSSSWYNV

SEQ ID NO: 164 - protein, 10 aa, Artificial Sequence
  humanized antibody
QCNYIIDYGA

SEQ ID NO: 165 - protein, 10 aa, Artificial Sequence
  humanized antibody
QSYYNSDSDA

SEQ ID NO: 166 - protein, 12 aa, Artificial Sequence
  humanized antibody
QQGYTEDNIDNT

SEQ ID NO: 167 - protein, 12 aa, Artificial Sequence
  humanized antibody
QGAVYSGNTEWA

SEQ ID NO: 168 - protein, 13 aa, Artificial Sequence
  humanized antibody
QGEFSCVSADCIA

SEQ ID NO: 169 - protein, 12 aa, Artificial Sequence
  humanized antibody
QCTYYDNNYGGA

SEQ ID NO: 170 - protein, 15 aa, Artificial Sequence
  humanized antibody
QSWYYSGSGSYHSWA

SEQ ID NO: 171 - protein, 107 aa, Homo sapiens [sequence omitted]

SEQ ID NO: 172 - protein, 329 aa, Homo sapiens
ASTKGPSVFPLAPSSKSTSGGTAALGCLVKDYFPEPVTVSWNSGALTSGVHTFPAVLQSSGLYSLSSVVTVPSSSLGTQTYICNVNHKPSNTKVDKKVEPKSCDKTHTCPPCPAPEAAGGPSVFLFPPKPKDTLMISRTPEVTCVVVDVSHEDPEVKFNWYVDGVEVHNAKTKPREEQYNSTYRVVSVLTVLHQDWLNGKEYKCKVSNKALPAPIEKTISKAKGQPREPQVYTLPPSREEMTKNQVSLTCLVKGFYPSDIAVEWESNGQPENNYKTTPPVLDSDGSFFLYSKLTVDKSRWQQGNVFSCSVMHEALHNHYTQKSLSLSPG

SEQ ID NO: 173 - protein, 123 aa, Artificial Sequence
  humanized antibody
EVQLLESGGRLVQPGTSLRLSCAVSGIDLSSYAMGWVRQAPGKGLEYVGVITSSATTYYASWAKGRFTISKTSSKNTLYLQMNSLRAEDTAVYFCARGGPGYSTNTHYAFDPWGQGTLVTVSS

SEQ ID NO: 174 - protein, 108 aa, Artificial Sequence
  Humanized antibody
DVQMTQSPSSLSASVGDRVTITCQASQSIYSFLSWYQQKPGQAPKLLIYAASDLESGVPSRFSGSGSGTDFTLTISSLQPEDFATYYCQSNYIIDYGAFGQGTKVVIK

SEQ ID NO: 175 - protein, 10 aa, Artificial Sequence
  Humanized antibody
QSNYIIDYGA